European Patent Application EP 4 201 956 A1, published June 28, 2023. Title: Site-specific antibody conjugation and its use. Applicant: F. Hoffmann-La Roche AG. The sequence listing filed with the application follows.

SEQUENCE LISTING (34 sequences)

SEQ ID NO: 1 - protein, 329 aa, Homo sapiens
ASTKGPSVFPLAPSSKSTSGGTAALGCLVKDYFPEPVTVSWNSGALTSGVHTFPAVLQSSGLYSLSSVVTVPSSSLGTQTYICNVNHKPSNTKVDKKVEPKSCDKTHTCPPCPAPELLGGPSVFLFPPKPKDTLMISRTPEVTCVVVDVSHEDPEVKFNWYVDGVEVHNAKTKPREEQYNSTYRVVSVLTVLHQDWLNGKEYKCKVSNKALPAPIEKTISKAKGQPREPQVYTLPPSRDELTKNQVSLTCLVKGFYPSDIAVEWESNGQPENNYKTTPPVLDSDGSFFLYSKLTVDKSRWQQGNVFSCSVMHEALHNHYTQKSLSLSPG

SEQ ID NO: 2 - protein, 329 aa, Homo sapiens
ASTKGPSVFPLAPSSKSTSGGTAALGCLVKDYFPEPVTVSWNSGALTSGVHTFPAVLQSSGLYSLSSVVTVPSSSLGTQTYICNVNHKPSNTKVDKKVEPKSCDKTHTCPPCPAPELLGGPSVFLFPPKPKDTLMISRTPEVTCVVVDVSHEDPEVKFNWYVDGVEVHNAKTKPREEQYNSTYRVVSVLTVLHQDWLNGKEYKCKVSNKALPAPIEKTISKAKGQPREPQVYTLPPSREEMTKNQVSLTCLVKGFYPSDIAVEWESNGQPENNYKTTPPVLDSDGSFFLYSKLTVDKSRWQQGNVFSCSVMHEALHNHYTQKSLSLSPG

SEQ ID NO: 3 - protein, 325 aa, Homo sapiens
ASTKGPSVFPLAPCSRSTSESTAALGCLVKDYFPEPVTVSWNSGALTSGVHTFPAVLQSSGLYSLSSVVTVPSSNFGTQTYTCNVDHKPSNTKVDKTVERKCCVECPPCPAPPVAGPSVFLFPPKPKDTLMISRTPEVTCVVVDVSHEDPEVQFNWYVDGVEVHNAKTKPREEQFNSTFRVVSVLTVVHQDWLNGKEYKCKVSNKGLPAPIEKTISKTKGQPREPQVYTLPPSREEMTKNQVSLTCLVKGFYPSDIAVEWESNGQPENNYKTTPPMLDSDGSFFLYSKLTVDKSRWQQGNVFSCSVMHEALHNHYTQKSLSLSPG

SEQ ID NO: 4 - protein, 376 aa, Homo sapiens
ASTKGPSVFPLAPCSRSTSGGTAALGCLVKDYFPEPVTVSWNSGALTSGVHTFPAVLQSSGLYSLSSVVTVPSSSLGTQTYTCNVNHKPSNTKVDKRVELKTPLGDTTHTCPRCPEPKSCDTPPPCPRCPEPKSCDTPPPCPRCPEPKSCDTPPPCPRCPAPELLGGPSVFLFPPKPKDTLMISRTPEVTCVVVDVSHEDPEVQFKWYVDGVEVHNAKTKPREEQYNSTFRVVSVLTVLHQDWLNGKEYKCKVSNKALPAPIEKTISKTKGQPREPQVYTLPPSREEMTKNQVSLTCLVKGFYPSDIAVEWESSGQPENNYNTTPPMLDSDGSFFLYSKLTVDKSRWQQGNIFSCSVMHEALHNRFTQKSLSLSPG

SEQ ID NO: 5 - protein, 326 aa, Homo sapiens
ASTKGPSVFPLAPCSRSTSESTAALGCLVKDYFPEPVTVSWNSGALTSGVHTFPAVLQSSGLYSLSSVVTVPSSSLGTKTYTCNVDHKPSNTKVDKRVSPNMVPHAHHAQAPEFLGGPSVFLFPPKPKDTLMISRTPEVTCVVVDVSQEDPEVQFNWYVDGVEVHNAKTKPREEQFNSTYRVVSVLTVLHQDWLNGKEYKCKVSNKGLPSSIEKTISKAKGQPREPQVYTLPPSQEEMTKNQVSLTCLVKGFYPSDIAVEWESNGQPENNYKTTPPVLDSDGSFFLYSRLTVDKSRWQEGNVFSCSVMHEALHNHYTQKSLSLSLG

SEQ ID NO: 6 - protein, 107 aa, Homo sapiens [sequence omitted]

SEQ ID NO: 7 - protein, 105 aa, Homo sapiens
QPKAAPSVTLFPPSSEELQANKATLVCLISDFYPGAVTVAWKADSSPVKAGVETTTPSKQSNNKYAASSYLSLTPEQWKSHRSYSCQVTHEGSTVEKTVAPTECS

SEQ ID NO: 8 - protein, 342 aa, Artificial Sequence
  Modified heavy chain-constant region
ASTKGPSVFPLAPSSKSTSGGTAALGCLVKDYFPEPVTVSWNSGALTSGVHTFPAVLQSSGLYSLSSVVTVPSSSLGTQTYICNVNHKPSNTKVDKKVEPKSCDKTHTCPPCPAPELLGGPSVFLFPPKPKDTLMISRTPEVTCVVVDVSHEDPEVKFNWYVDGVEVHNAKTKPREEQYNGGGSYRYRQGGGSSTYRVVSVLTVLHQDWLNGKEYKCKVSNKALPAPIEKTISKAKGQPREPQVYTLPPSRDELTKNQVSLTCLVKGFYPSDIAVEWESNGQPENNYKTTPPVLDSDGSFFLYSKLTVDKSRWQQGNVFSCSVMHEALHNHYTQKSLSLSPG

SEQ ID NO: 9 - protein, 342 aa, Artificial Sequence
  Modified heavy chain-constant region
ASTKGPSVFPLAPSSKSTSGGTAALGCLVKDYFPEPVTVSWNSGALTSGVHTFPAVLQSSGLYSLSSVVTVPSSSLGTQTYICNVNHKPSNTKVDKKVEPKSCDKTHTCPPCPAPELLGGPSVFLFPPKPKDTLMISRTPEVTCVVVDVSHEDPEVKFNWYVDGVEVHNAKTKPREEQYNSTYRVVSVLTVLHQDWLNGKEYKCKVSNKALPAPIEKTISKAKGGGGSYRYRQGGGSQPREPQVYTLPPSRDELTKNQVSLTCLVKGFYPSDIAVEWESNGQPENNYKTTPPVLDSDGSFFLYSKLTVDKSRWQQGNVFSCSVMHEALHNHYTQKSLSLSPG

SEQ ID NO: 10 - protein, 120 aa, Artificial Sequence
  Modified light chain-constant region
RTVAAPSVFIFPPSDEQLKSGTASVVCLLNNFYPREAKVQWKVDNALQSGNSQESVTEQDSKDSTYSLSSTLTLSKADYEKHKVYACEVTHQGLSSPVTKSFNRGECGGGSYRYRQGGGS

SEQ ID NO: 11 - protein, 5 aa, Artificial Sequence
  Q-tag
RYGQR

SEQ ID NO: 12 - protein, 5 aa, Artificial Sequence
  Q-tag
RWRQR

SEQ ID NO: 13 - protein, 5 aa, Artificial Sequence
  Q-tag
YRQRT

SEQ ID NO: 14 - protein, 5 aa, Artificial Sequence
  Q-tag
IRQRQ

SEQ ID NO: 15 - protein, 5 aa, Artificial Sequence
  Q-tag
FRYRQ

SEQ ID NO: 16 - protein, 5 aa, Artificial Sequence
  K-tag
RYESK

SEQ ID NO: 17 - protein, 5 aa, Artificial Sequence
  Q-tag
YRYRQ

SEQ ID NO: 18 - protein, 5 aa, Artificial Sequence
  Q-tag
RVRQR

SEQ ID NO: 19 - protein, 4 aa, Artificial Sequence
  Linker
GGGS

SEQ ID NO: 20 - protein, 4 aa, Artificial Sequence
  Linker
GGGP

SEQ ID NO: 21 - protein, 4 aa, Artificial Sequence
  Linker
ESGS

SEQ ID NO: 22 - protein, 4 aa, Artificial Sequence
  Linker
APAP

SEQ ID NO: 23 - protein, 18 aa, Artificial Sequence
  KESGSVSSEQLAQFRSLD
KESGSVSSEQLAQFRSLD

SEQ ID NO: 24 - protein, 14 aa, Artificial Sequence
  Linker
EGKSSGSGSESKST

SEQ ID NO: 25 - protein, 13 aa, Artificial Sequence
  Q-tag motif with two flexible linkers
GGGSYRYRQGGGS

SEQ ID NO: 26 - protein, 13 aa, Artificial Sequence
  Q-tag motif with two flexible linkers
GGGSRVRQRGGGS

SEQ ID NO: 27 - protein, 343 aa, Artificial Sequence
  Modified heavy chain constant region
ASTKGPSVFPLAPSSKSTSGGTAALGCLVKDYFPEPVTVSWNSGALTSGVHTFPAVLQSSGGGSYRYRQGGGSGLYSLSSVVTVPSSSLGTQTYICNVNHKPSNTKVDKKVEPKSCDKTHTCPPCPAPEAAGGPSVFLFPPKPKDTLMISRTPEVTCVVVDVSHEDPEVKFNWYVDGVEVHNAKTKPREEQYNSTYRVVSVLTVLHQDWLNGKEYKCKVSNKALGAPIEKTISKAKGQPREPQVYTLPPSREEMTKNQVSLTCLVKGFYPSDIAVEWESNGQPENNYKTTPPVLDSDGSFFLYSKLTVDKSRWQQGNVFSCSVMHEALHNHYTQKSLSLSPGK

SEQ ID NO: 28 - protein, 343 aa, Artificial Sequence
  Modified heavy chain constant region
ASTKGPSVFPLAPSSKSTSGGTAALGCLVKDYFPEPVTVSWNSGALTSGVHTFPAVLQSSGLYSLSSVVTVPSSSLGTQTYICNVNHKPSNTKVDKKVEPKSCDKTHTCPPCPAPEAAGGPSVFLFPPKPKDTLMISRTPEVTCVVVDVSHEDPEVKFNWYVDGVEVHNAKTKPREEQYNSTYRVVSVLTVLHQDWLNGKEYKCKVSNKALGAPIEKTISKAKGQPREPQVYTLPPSREEMTKNQVSLTCLVKGFYPSDIAVEWESNGQPENNYKTTPPVLDSDGGGSYRYRQGGGSGSFFLYSKLTVDKSRWQQGNVFSCSVMHEALHNHYTQKSLSLSPGK

SEQ ID NO: 29 - protein, 107 aa, Artificial Sequence [sequence omitted]

SEQ ID NO: 30 - protein, 107 aa, Artificial Sequence [sequence omitted]

SEQ ID NO: 31 - protein, 262 aa, Kutzneria albida
MHKWFLRAAVVAAVGFGLPTLIATTAQAAAVAAPTPRAPLAPPLAEDRSYRTWRVEDYVEAWERYHGREMTEDERENLARGCIGVTVVNLNREDLSNPPLNLSFGSLRTAEAVQAALNKIVDTHPSPAQYEAAVAKDPILKRLKNVVKALPSWIDSAKLKASIFSKRFYSWQNPDWSEERAHTTYRPDRETDQVDMSTYRYRARPGYVNFDYGWFDQDTNTWWHANHEEPRMVVYQSTLRHYSRPLQDFDEQVFTVAFAKKD

SEQ ID NO: 32 - protein, 240 aa, Artificial Sequence
  Fc-region including part of the hinge region with a first recognition site
DKTHTCPPCPAPEAAGGPSVFLFPPKPKDTLMISRTPEVTCVVVDVSHEDPEVKFNWYVDGVEVHNAKTKPREEQYNSTYRVVSVLTVLHQDWLNGKEYKCKVSNKALGAPIEKTISKAKGQPREPQVYTLPPSREEMTKNQVSLTCLVKGFYPSDIAVEWESNGQPENNYKTTPPVLDSDGGGSYRYRQGGGSGSFFLYSKLTVDKSRWQQGNVFSCSVMHEALHNHYTQKSLSLSPGK

SEQ ID NO: 33 - protein, 227 aa, Artificial Sequence
  Fc-region including part of the hinge region without a first recognition site
DKTHTCPPCPAPEAAGGPSVFLFPPKPKDTLMISRTPEVTCVVVDVSHEDPEVKFNWYVDGVEVHNAKTKPREEQYNSTYRVVSVLTVLHQDWLNGKEYKCKVSNKALGAPIEKTISKAKGQPREPQVYTLPPSREEMTKNQVSLTCLVKGFYPSDIAVEWESNGQPENNYKTTPPVLDSDGSFFLYSKLTVDKSRWQQGNVFSCSVMHEALHNHYTQKSLSLSPGK

SEQ ID NO: 34 - protein, 342 aa, Artificial Sequence
  Modified heavy chain-constant region
ASTKGPSVFPLAPSSKSTSGGTAALGCLVKDYFPEPVTVSWNSGALTSGVHTFPAVLQSSGGGSYRYRQGGGSGLYSLSSVVTVPSSSLGTQTYICNVNHKPSNTKVDKKVEPKSCDKTHTCPPCPAPELLGGPSVFLFPPKPKDTLMISRTPEVTCVVVDVSHEDPEVKFNWYVDGVEVHNAKTKPREEQYNSTYRVVSVLTVLHQDWLNGKEYKCKVSNKALPAPIEKTISKAKGQPREPQVYTLPPSRDELTKNQVSLTCLVKGFYPSDIAVEWESNGQPENNYKTTPPVLDSDGSFFLYSKLTVDKSRWQQGNVFSCSVMHEALHNHYTQKSLSLSPG